European Patent Application EP 4 372 091 A2, published May 22, 2024. Title: COMPOSITIONS AND METHODS FOR EDITING NUCLEIC ACIDS IN CELLS UTILIZING OLIGONUCLEOTIDES. Applicant: WOOLF, Tod M. The sequence listing filed with the application follows.

SEQUENCE LISTING (110 sequences)

SEQ ID NO: 1 - DNA, 72 bp, synthetic construct
  misc_feature 1..72: note = Synthetic oligonucleotide (ETAGEN Serial Number 100001)
  misc_feature 1..72: note = Base modification: 3 phosphorothioates end-blocks on each terminus
  source 1..72: mol_type = other DNA
catgtggtcggggtagcggctgaagcactgcacgccgtaggtcagggtggtcacgagggtgggccagggcac

SEQ ID NO: 2 - DNA, 72 bp, synthetic construct
  misc_feature 1..72: note = Synthetic oligonucleotide (ETAGEN Serial Number 100002)
  misc_feature 1..72: note = Base modification: 3 phosphorothioates end-blocks on each terminus
  source 1..72: mol_type = other DNA
catgtggtcggggtagcggctgaagcactgcacgccctaggtcagggtggtcacgagggtgggccagggcac

SEQ ID NO: 3 - DNA, 40 bp, synthetic construct
  misc_feature 1..40: note = Synthetic oligonucleotide (ETAGEN Serial Number 100003)
  source 1..40: mol_type = other DNA
cggctgaagcactgcacgccgtaggtcagggtggtcacga

SEQ ID NO: 4 - DNA, 40 bp, synthetic construct
  misc_feature 1..40: note = Synthetic oligonucleotide (ETAGEN Serial Number 100004)
  source 1..40: mol_type = other DNA
cggctgaagcactgcacgccctaggtcagggtggtcacga

SEQ ID NO: 5 - DNA, 40 bp, synthetic construct; identical to SEQ ID NO: 3
  misc_feature 1..40: note = Synthetic oligonucleotide (ETAGEN Serial Number 100005)
  misc_feature 1..40: note = Base modification: 3 phosphorothioates end-blocks on each terminus (Parent)
  source 1..40: mol_type = other DNA

SEQ ID NO: 6 - DNA, 40 bp, synthetic construct; identical to SEQ ID NO: 4
  misc_feature 1..40: note = Synthetic oligonucleotide (ETAGEN Serial Number 100006)
  misc_feature 1..40: note = Base modification: 3 phosphorothioates end-blocks on each terminus
  source 1..40: mol_type = other DNA

SEQ ID NO: 7 - DNA, 40 bp, synthetic construct; identical to SEQ ID NO: 3
  misc_feature 1..40: note = Synthetic oligonucleotide (ETAGEN Serial Number 100007)
  misc_feature 1..40: note = Base modification: half phosphorothioates positive 40 mer (9s-20o-10s) with unmodified editing region
  source 1..40: mol_type = other DNA

SEQ ID NO: 8 - DNA, 40 bp, synthetic construct; identical to SEQ ID NO: 4
  misc_feature 1..40: note = Synthetic oligonucleotide (ETAGEN Serial Number 100008)
  misc_feature 1..40: note = Base modification: half phosphorothioates positive 40 mer (9s-20o-10s) with unmodified editing region
  source 1..40: mol_type = other DNA

SEQ ID NO: 9 - DNA, 40 bp, synthetic construct
  misc_feature 1..40: note = Synthetic oligonucleotide (ETAGEN Serial Number 100009)
  misc_feature 1..40: note = Base modification: half phosphorothioates positive 40 mer (9s-20o-10s) with unmodified editing region
  source 1..40: mol_type = other DNA
ctgcgagatcgcggcagcgccatgctgaggctcgtacaga

SEQ ID NO: 10 - DNA, 40 bp, synthetic construct; identical to SEQ ID NO: 3
  misc_feature 1..40: note = Synthetic oligonucleotide (ETAGEN Serial Number 100010)
  misc_feature 1..40: note = Base modification: Majority phosphorothiotes except in editing region (16s-6o-17s)
  source 1..40: mol_type = other DNA

SEQ ID NO: 11 - DNA, 40 bp, synthetic construct; identical to SEQ ID NO: 4
  misc_feature 1..40: note = Synthetic oligonucleotide (ETAGEN Serial Number 100011)
  misc_feature 1..40: note = Base modification: Majority phosphorothiotes except in editing region (16s-6o-17s)
  source 1..40: mol_type = other DNA

SEQ ID NO: 12 - DNA, 40 bp, synthetic construct; identical to SEQ ID NO: 9
  misc_feature 1..40: note = Synthetic oligonucleotide (ETAGEN Serial Number 100012)
  misc_feature 1..40: note = Base modification: Majority phosphorothiotes except in editing region (16s-6o-17s)
  source 1..40: mol_type = other DNA

SEQ ID NO: 13 - DNA, 40 bp, synthetic construct; identical to SEQ ID NO: 3
  misc_feature 1..40: note = Synthetic oligonucleotide (ETAGEN Serial Number 100013)
  misc_feature 1..40: note = Base modification: 3' 8x2'F high affinity arms with s end-blocks
  source 1..40: mol_type = other DNA

SEQ ID NO: 14 - DNA, 40 bp, synthetic construct; identical to SEQ ID NO: 4
  misc_feature 1..40: note = Synthetic oligonucleotide (ETAGEN Serial Number 100014)
  misc_feature 1..40: note = Base modification: 3' 8x2'F high affinity arms with s end-blocks
  source 1..40: mol_type = other DNA

SEQ ID NO: 15 - DNA, 42 bp, synthetic construct
  misc_feature 1..42: note = Synthetic oligonucleotide (ETAGEN Serial Number 100015)
  misc_feature 1..42: note = Base modification: 5' non-phosphorothioate end-block (methyphosphonate), 3' 3s end-blocks
  source 1..42: mol_type = other DNA
ttcggctgaagcactgcacgccgtaggtcagggtggtcacga

SEQ ID NO: 16 - DNA, 42 bp, synthetic construct
  misc_feature 1..42: note = Synthetic oligonucleotide (ETAGEN Serial Number 100016)
  misc_feature 1..42: note = Base modification: 5' non-phosphorothioate end-block (methyphosphonate), 3' 3s end-blocks
  source 1..42: mol_type = other DNA
ttcggctgaagcactgcacgccctaggtcagggtggtcacga

SEQ ID NO: 17 - DNA, 40 bp, synthetic construct; identical to SEQ ID NO: 3
  misc_feature 1..40: note = Synthetic oligonucleotide (ETAGEN Serial Number 100017)
  misc_feature 1..40: note = Base modification: C's replaced with 5' methyl C to fool repair machinery, as to which strand is nascent
  source 1..40: mol_type = other DNA

SEQ ID NO: 18 - DNA, 40 bp, synthetic construct; identical to SEQ ID NO: 4
  misc_feature 1..40: note = Synthetic oligonucleotide (ETAGEN Serial Number 100018)
  misc_feature 1..40: note = Base modification: C's replaced with 5' methyl C to fool repair machinery, as to which strand is nascent
  source 1..40: mol_type = other DNA

SEQ ID NO: 19 - RNA, 13 nt, synthetic construct
  misc_feature 1..13: note = Synthetic oligonucleotide (ETAGEN Serial Number 100019)
  misc_feature 1..13: note = Base modification: 2' -O-methyl "protector" oligo complimentary to positions 1-13 of editing oligo
  source 1..13: mol_type = other RNA
agtgcttcagccg

SEQ ID NO: 20 - RNA, 14 nt, synthetic construct
  misc_feature 1..14: note = Synthetic oligonucleotide (ETAGEN Serial Number 100020)
  misc_feature 1..14: note = Base modification: 2' -O-methyl "protector" oligo complimentary to positions 14-27 of editing oligo
  source 1..14: mol_type = other RNA
gacctacggcgtgc

SEQ ID NO: 21 - RNA, 13 nt, synthetic construct
  misc_feature 1..13: note = Synthetic oligonucleotide (ETAGEN Serial Number 100021)
  misc_feature 1..13: note = Base modification: 2' -O-methyl "protector" oligo complimentary to positions 28-40 of editing oligo
  source 1..13: mol_type = other RNA
tcgtgaccaccct

SEQ ID NO: 22 - DNA, 25 bp, synthetic construct
  misc_feature 1..25: note = Synthetic oligonucleotide (ETAGEN Serial Number 100022)
  misc_feature 1..25: note = Base modification: 25mer all phosphorothioate DNA
  source 1..25: mol_type = other DNA
gcactgcacgccctaggtcagggtg

SEQ ID NO: 23 - DNA, 25 bp, synthetic construct
  misc_feature 1..25: note = Synthetic oligonucleotide (ETAGEN Serial Number 100023)
  misc_feature 1..25: note = Base modification: 25mer all phosphorothioate DNA
  source 1..25: mol_type = other DNA
gcactgcacgccgtaggtcagggtg

SEQ ID NO: 24 - DNA, 25 bp, synthetic construct
  misc_feature 1..25: note = Synthetic oligonucleotide (ETAGEN Serial Number 100024)
  misc_feature 1..25: note = Base modification: 25mer all phosphorothioate DNA
  source 1..25: mol_type = other DNA
tcgcggcagcgccatgctgaggatc

SEQ ID NO: 25 - DNA, 40 bp, synthetic construct; identical to SEQ ID NO: 3
  misc_feature 1..40: note = Synthetic oligonucleotide (ETAGEN Serial Number 100031)
  misc_feature 1..40: note = Base modification: 3 phosphorothioates end-blocks on each terminus (PARENT)
  source 1..40: mol_type = other DNA

SEQ ID NO: 26 - DNA, 40 bp, synthetic construct; identical to SEQ ID NO: 4
  misc_feature 1..40: note = Synthetic oligonucleotide (ETAGEN Serial Number 100032)
  misc_feature 1..40: note = Base modification: 40mers (with 3 phosphorothioates on each terminus)
  source 1..40: mol_type = other DNA

SEQ ID NO: 27 - DNA, 40 bp, synthetic construct; identical to SEQ ID NO: 4
  misc_feature 1..40: note = Synthetic oligonucleotide (ETAGEN Serial Number 100033)
  misc_feature 1..40: note = Base modification: 5' and 3' 8x2'F high affinity arms with s end-blocks
  source 1..40: mol_type = other DNA

SEQ ID NO: 28 - DNA, 40 bp, synthetic construct; identical to SEQ ID NO: 3
  misc_feature 1..40: note = Synthetic oligonucleotide (ETAGEN Serial Number 100034)
  misc_feature 1..40: note = Base modification: 5' and 3' 8x2'F high affinity arms with s end-blocks
  source 1..40: mol_type = other DNA

SEQ ID NO: 29 - DNA, 40 bp, synthetic construct; identical to SEQ ID NO: 3
  misc_feature 1..40: note = Synthetic oligonucleotide (ETAGEN Serial Number 100035)
  misc_feature 1..40: note = Base modification: 3' 8x2'-O-methyl high affinity arms with s end-blocks
  source 1..40: mol_type = other DNA

SEQ ID NO: 30 - DNA, 40 bp, synthetic construct; identical to SEQ ID NO: 4
  misc_feature 1..40: note = Synthetic oligonucleotide (ETAGEN Serial Number 100036)
  misc_feature 1..40: note = Base modification: 3' 8x2'-O-methyl high affinity arms with s end-blocks
  source 1..40: mol_type = other DNA

SEQ ID NO: 31 - DNA, 40 bp, synthetic construct; identical to SEQ ID NO: 3
  misc_feature 1..40: note = Synthetic oligonucleotide (ETAGEN Serial Number 100037)
  misc_feature 1..40: note = Base modification: 5' 8x2'-O-methyl high affinity arms with s end-blocks
  source 1..40: mol_type = other DNA

SEQ ID NO: 32 - DNA, 40 bp, synthetic construct; identical to SEQ ID NO: 4
  misc_feature 1..40: note = Synthetic oligonucleotide (ETAGEN Serial Number 100038)
  misc_feature 1..40: note = Base modification: 5' 8x2'-O-methyl high affinity arms with s end-blocks
  source 1..40: mol_type = other DNA

SEQ ID NO: 33 - DNA, 40 bp, synthetic construct; identical to SEQ ID NO: 4
  misc_feature 1..40: note = Synthetic oligonucleotide (ETAGEN Serial Number 100039)
  misc_feature 1..40: note = Base modification: 5' and 3' 8x2'-O-methyl high affinity arms with s end-blocks
  source 1..40: mol_type = other DNA

SEQ ID NO: 34 - DNA, 40 bp, synthetic construct; identical to SEQ ID NO: 3
  misc_feature 1..40: note = Synthetic oligonucleotide (ETAGEN Serial Number 100040)
  misc_feature 1..40: note = Base modification: 5' and 3' 8x2'-O-methyl high affinity arms with s end-blocks
  source 1..40: mol_type = other DNA

SEQ ID NO: 35 - DNA, 40 bp, synthetic construct; identical to SEQ ID NO: 4
  misc_feature 1..40: note = Synthetic oligonucleotide (ETAGEN Serial Number 100041)
  misc_feature 1..40: note = Base modification: Central C's replaced with 5' methyl C to fool repair machinery as to which strand is nascent
  source 1..40: mol_type = other DNA

SEQ ID NO: 36 - DNA, 40 bp, synthetic construct; identical to SEQ ID NO: 3
  misc_feature 1..40: note = Synthetic oligonucleotide (ETAGEN Serial Number 100042)
  misc_feature 1..40: note = Base modification: Central C's replaced with 5' methyl C to fool repair machinery as to which strand is nascent
  source 1..40: mol_type = other DNA

SEQ ID NO: 37 - DNA, 40 bp, synthetic construct; identical to SEQ ID NO: 3
  misc_feature 1..40: note = Synthetic oligonucleotide (ETAGEN Serial Number 100043)
  misc_feature 1..40: note = Base modification: Central C replaced with 5' methyl C to fool repair machinery as to which strand is nascent
  source 1..40: mol_type = other DNA

SEQ ID NO: 38 - DNA, 40 bp, synthetic construct; identical to SEQ ID NO: 4
  misc_feature 1..40: note = Synthetic oligonucleotide (ETAGEN Serial Number 100044)
  misc_feature 1..40: note = Base modification: Central C replaced with 5' methyl C to fool repair machinery as to which strand is nascent
  source 1..40: mol_type = other DNA

SEQ ID NO: 39 - DNA, 44 bp, synthetic construct
  misc_feature 1..44: note = Synthetic oligonucleotide (ETAGEN Serial Number 100045)
  misc_feature 1..44: note = Base modification: Phosphorothiote-free methylphosphonoate end-blocks, 5 methyl C's and 2'F arms
  source 1..44: mol_type = other DNA
ttcggctgaagcactgcacgccgtaggtcagggtggtcacgatt

SEQ ID NO: 40 - DNA, 42 bp, synthetic construct; identical to SEQ ID NO: 15
  misc_feature 1..42: note = Synthetic oligonucleotide (ETAGEN Serial Number 100047)
  misc_feature 1..42: note = Base modification: 5' methylphosphonoate end-blocks, 3' s-end-blocks, 5 methyl C's and 3' 2'F arm
  source 1..42: mol_type = other DNA

SEQ ID NO: 41 - DNA, 42 bp, synthetic construct; identical to SEQ ID NO: 16
  misc_feature 1..42: note = Synthetic oligonucleotide (ETAGEN Serial Number 100048)
  misc_feature 1..42: note = Base modification: 5' methylphosphonoate end-blocks, 3' s-end-blocks, 5 methyl C's and 3' 2'F arm
  source 1..42: mol_type = other DNA

SEQ ID NO: 42 - DNA, 44 bp, synthetic construct
  misc_feature 1..44: note = Synthetic oligonucleotide (ETAGEN Serial Number 100049)
  misc_feature 1..44: note = Base modification: Phosphorothioate-free 5' and 3' methylphosphonate end-blocks
  source 1..44: mol_type = other DNA
ttcggctgaagcactgcacgccctaggtcagggtggtcacgatt

SEQ ID NO: 43 - DNA, 44 bp, synthetic construct; identical to SEQ ID NO: 39
  misc_feature 1..44: note = Synthetic oligonucleotide (ETAGEN Serial Number 100050)
  misc_feature 1..44: note = Base modification: Phosphorothioate-free 5' and 3' methylphosphonate end-blocks
  source 1..44: mol_type = other DNA

SEQ ID NO: 44 - DNA, 40 bp, synthetic construct; identical to SEQ ID NO: 3
  misc_feature 1..40: note = Synthetic oligonucleotide (ETAGEN Serial Number 100058)
  misc_feature 1..40: note = Base modification: 5' 8x2'-O-methyl and 8x3' 2'F high affinity arms with s end-blocks
  source 1..40: mol_type = other DNA

SEQ ID NO: 45 - DNA, 40 bp, synthetic construct; identical to SEQ ID NO: 3
  misc_feature 1..40: note = Synthetic oligonucleotide (ETAGEN Serial Number 100060)
  misc_feature 1..40: note = Base modification: 5' 8x2'-O-methyl and 3' 8x2'F high affinity arms with s end-blocks, with central 5 Methyl Cs
  source 1..40: mol_type = other DNA

SEQ ID NO: 46 - DNA, 40 bp, synthetic construct; identical to SEQ ID NO: 3
  misc_feature 1..40: note = Synthetic oligonucleotide (ETAGEN Serial Number 100062)
  misc_feature 1..40: note = Base modification: 3' 14x2'F high affinity arms with s end-blocks
  source 1..40: mol_type = other DNA

SEQ ID NO: 47 - DNA, 40 bp, synthetic construct; identical to SEQ ID NO: 3
  misc_feature 1..40: note = Synthetic oligonucleotide (ETAGEN Serial Number 100064)
  misc_feature 1..40: note = Base modification: 3' 20x2'F high affinity arms with s end-blocks
  source 1..40: mol_type = other DNA

SEQ ID NO: 48 - DNA, 40 bp, synthetic construct; identical to SEQ ID NO: 3
  misc_feature 1..40: note = Synthetic oligonucleotide (ETAGEN Serial Number 100066)
  misc_feature 1..40: note = Base modification: 5' 14x2'-O-methyl high affinity arms with s end-blocks
  source 1..40: mol_type = other DNA

SEQ ID NO: 49 - DNA, 40 bp, synthetic construct; identical to SEQ ID NO: 3
  misc_feature 1..40: note = Synthetic oligonucleotide (ETAGEN Serial Number 100068)
  misc_feature 1..40: note = Base modification: 5' 20x2'-O-methyl high affinity arms with s end-blocks
  source 1..40: mol_type = other DNA

SEQ ID NO: 50 - DNA, 72 bp, synthetic construct; identical to SEQ ID NO: 1
  misc_feature 1..72: note = Synthetic oligonucleotide (ETAGEN Serial Number 100070)
  misc_feature 1..72: note = Base modification: 5' 8x2'-O-methyl high affinity arms with s end-blocks
  source 1..72: mol_type = other DNA

SEQ ID NO: 51 - DNA, 72 bp, synthetic construct; identical to SEQ ID NO: 1
  misc_feature 1..72: note = Synthetic oligonucleotide (ETAGEN Serial Number 100072)
  misc_feature 1..72: note = Base modification: 5' 24x2'-O-methyl high affinity arms with s end-blocks
  source 1..72: mol_type = other DNA

SEQ ID NO: 52 - DNA, 44 bp, synthetic construct
  misc_feature 1..44: note = Synthetic oligonucleotide (ETAGEN Serial Number 100074)
  misc_feature 1..44: note = Base modification: end-block 3' phosphorothioate end-block
  source 1..44: mol_type = other DNA
cggctgaagcactgcacgccgtaggtcagggtggtcacgacgcg

SEQ ID NO: 53 - DNA, 40 bp, synthetic construct; identical to SEQ ID NO: 3
  misc_feature 1..40: note = Synthetic oligonucleotide (ETAGEN Serial Number 100076)
  misc_feature 1..40: note = Base modification: amino linker (TriLink Biotechnologies, San Diego, CA) end-blocks
  source 1..40: mol_type = other DNA

SEQ ID NO: 54 - DNA, 40 bp, synthetic construct; identical to SEQ ID NO: 3
  misc_feature 1..40: note = Synthetic oligonucleotide (ETAGEN Serial Number 100078)
  misc_feature 1..40: note = Base modification: 5' and 3' end-blocks
  source 1..40: mol_type = other DNA

SEQ ID NO: 55 - DNA, 40 bp, synthetic construct; identical to SEQ ID NO: 3
  misc_feature 1..40: note = Synthetic oligonucleotide (ETAGEN Serial Number 100079)
  misc_feature 1..40: note = Base modification: amino linkers 5' and 3' end-blocks (TriLink Biotechnologies, San Diego, CA)
  source 1..40: mol_type = other DNA

SEQ ID NO: 56 - DNA, 40 bp, synthetic construct; identical to SEQ ID NO: 3
  misc_feature 1..40: note = Synthetic oligonucleotide (ETAGEN Serial Number 100080)
  misc_feature 1..40: note = Base modification: Amino Linker end-blocks with 3' 10x2'F arm 5' 11x2'-O-methyl and 5 Methyl C editing region
  source 1..40: mol_type = other DNA

SEQ ID NO: 57 - DNA, 40 bp, synthetic construct
  misc_feature 1..40: note = Synthetic oligonucleotide (ETAGEN Serial Number 100082)
  misc_feature 1..40: note = Base modification: COMPLEMENTARY DNA STRAND TO THE PARENT with phosphorothioate end-blocks
  source 1..40: mol_type = other DNA
tcgtgaccaccctgacctacggcgtgcagtgcttcagccg

SEQ ID NO: 58 - DNA, 40 bp, synthetic construct; identical to SEQ ID NO: 57
  misc_feature 1..40: note = Synthetic oligonucleotide (ETAGEN Serial Number 100083)
  misc_feature 1..40: note = Base modification: COMPLEMENTARY RNA STRAND TO THE PARENT with phosphorothioate end-blocks
  source 1..40: mol_type = other DNA

SEQ ID NO: 59 - DNA, 40 bp, synthetic construct; identical to SEQ ID NO: 3
  misc_feature 1..40: note = Synthetic oligonucleotide (ETAGEN Serial Number 100084)
  misc_feature 1..40: note = Base modification: 5' 8xRNA and 3' 8x2'F high affinity arms with s end-blocks
  source 1..40: mol_type = other DNA

SEQ ID NO: 60 - DNA, 72 bp, synthetic construct; identical to SEQ ID NO: 1
  misc_feature 1..72: note = Synthetic oligonucleotide (ETAGEN Serial Number 100085)
  misc_feature 1..72: note = Base modification: Editing/Guide Strand with 5' RISC entry site of alternating RNA/2'-O-methyl
  source 1..72: mol_type = other DNA

SEQ ID NO: 61 - DNA, 21 bp, synthetic construct
  misc_feature 1..21: note = Synthetic oligonucleotide (ETAGEN Serial Number 100086)
  misc_feature 1..21: note = Base modification: Sense strand that will allow the duplex with 100085 to form editing compound capable of RISC entry
  source 1..21: mol_type = other DNA
ccgctaccccgaccacatgtt

SEQ ID NO: 62 - DNA, 71 bp, synthetic construct
  misc_feature 1..71: note = Synthetic oligonucleotide (Primary Indication: Alzheimer's Disease; Target: APP)
  source 1..71: mol_type = other DNA
tcaagacggaggagatctctgaagtgaagatggatgcagaattccgacatgactcaggatatgaagttcat

SEQ ID NO: 63 - DNA, 71 bp, synthetic construct
  misc_feature 1..71: note = Synthetic oligonucleotide (Primary Indication: Alzheimer's Disease; Target: APP)
  source 1..71: mol_type = other DNA
atgaacttcatatcctgagtcatgtcggaattctgcatccatcttcacttcagagatctcctccgtcttga

SEQ ID NO: 64 - DNA, 41 bp, synthetic construct
  misc_feature 1..41: note = Synthetic oligonucleotide (Primary Indication: Alzheimer's Disease; Target: APP)
  source 1..41: mol_type = other DNA
tctctgaagtgaagatggatgcagaattccgacatgactca

SEQ ID NO: 65 - DNA, 41 bp, synthetic construct
  misc_feature 1..41: note = Synthetic oligonucleotide (Primary Indication: Alzheimer's Disease; Target: APP)
  source 1..41: mol_type = other DNA
tgagtcatgtcggaattctgcatccatcttcacttcagaga

SEQ ID NO: 66 - DNA, 71 bp, synthetic construct
  misc_feature 1..71: note = Synthetic oligonucleotide (Primary Indication: Alzheimer's Disease; Target: APP)
  source 1..71: mol_type = other DNA
tcaagacggaggagatctctgaagtgaagatggatacagaattccgacatgactcaggatatgaagttcat

SEQ ID NO: 67 - DNA, 71 bp, synthetic construct
  misc_feature 1..71: note = Synthetic oligonucleotide (Primary Indication: Alzheimer's Disease; Target: APP)
  source 1..71: mol_type = other DNA
atgaacttcatatcctgagtcatgtcggaattctgtatccatcttcacttcagagatctcctccgtcttga

SEQ ID NO: 68 - DNA, 41 bp, synthetic construct
  misc_feature 1..41: note = Synthetic oligonucleotide (Primary Indication: Alzheimer's Disease; Target: APP)
  source 1..41: mol_type = other DNA
tctctgaagtgaagatggatacagaattccgacatgactca

SEQ ID NO: 69 - DNA, 41 bp, synthetic construct
  misc_feature 1..41: note = Synthetic oligonucleotide (Primary Indication: Alzheimer's Disease; Target: APP)
  source 1..41: mol_type = other DNA
tgagtcatgtcggaattctgtatccatcttcacttcagaga

SEQ ID NO: 70 - DNA, 71 bp, synthetic construct
  misc_feature 1..71: note = Synthetic oligonucleotide (Primary Indication: Alzheimer's Disease; Target: APOE)
  source 1..71: mol_type = other DNA
cgcaggcccggctgggcgcggacatggaggacgtgtgcggccgcctggtgcagtaccgcggcgaggtgcag

SEQ ID NO: 71 - DNA, 71 bp, synthetic construct
  misc_feature 1..71: note = Synthetic oligonucleotide (Primary Indication: Alzheimer's Disease; Target: APOE)
  source 1..71: mol_type = other DNA
ctgcacctcgccgcggtactgcaccaggcggccgcacacgtcctccatgtccgcgcccagccgggcctgcg

SEQ ID NO: 72 - DNA, 41 bp, synthetic construct
  misc_feature 1..41: note = Synthetic oligonucleotide (Primary Indication: Alzheimer's Disease; Target: APOE)
  source 1..41: mol_type = other DNA
gcgcggacatggaggacgtgtgcggccgcctggtgcagtac

SEQ ID NO: 73 - DNA, 41 bp, synthetic construct
  misc_feature 1..41: note = Synthetic oligonucleotide (Primary Indication: Alzheimer's Disease; Target: APOE)
  source 1..41: mol_type = other DNA
gtactgcaccaggcggccgcacacgtcctccatgtccgcgc

SEQ ID NO: 74 - DNA, 71 bp, synthetic construct
  misc_feature 1..71: note = Synthetic oligonucleotide (Primary Indication: Alzheimer's Disease; Target: APOE)
  source 1..71: mol_type = other DNA
agcggctcctccgcgatgccgatgacctgcagaagcgcctggcagtgtaccaggccggggcccgcgagggc

SEQ ID NO: 75 - DNA, 71 bp, synthetic construct
  misc_feature 1..71: note = Synthetic oligonucleotide (Primary Indication: Alzheimer's Disease; Target: APOE)
  source 1..71: mol_type = other DNA
gccctcgcgggccccggcctggtacactgccaggcgcttctgcaggtcatcggcatcgcggaggagccgct

SEQ ID NO: 76 - DNA, 41 bp, synthetic construct
  misc_feature 1..41: note = Synthetic oligonucleotide (Primary Indication: Alzheimer's Disease; Target: APOE)
  source 1..41: mol_type = other DNA
atgccgatgacctgcagaagcgcctggcagtgtaccaggcc

SEQ ID NO: 77 - DNA, 41 bp, synthetic construct
  misc_feature 1..41: note = Synthetic oligonucleotide (Primary Indication: Alzheimer's Disease; Target: APOE)
  source 1..41: mol_type = other DNA
ggcctggtacactgccaggcgcttctgcaggtcatcggcat

SEQ ID NO: 78 - DNA, 71 bp, synthetic construct
  misc_feature 1..71: note = Synthetic oligonucleotide (Primary Indication: Alzheimer's Disease; Target: APOE)
  source 1..71: mol_type = other DNA
agcggctcctccgcgatgccgatgacctgcagaagtgcctggcagtgtaccaggccggggcccgcgagggc

SEQ ID NO: 79 - DNA, 71 bp, synthetic construct
  misc_feature 1..71: note = Synthetic oligonucleotide (Primary Indication: Alzheimer's Disease; Target: APOE)
  source 1..71: mol_type = other DNA
gccctcgcgggccccggcctggtacactgccaggcacttctgcaggtcatcggcatcgcggaggagccgct

SEQ ID NO: 80 - DNA, 41 bp, synthetic construct
  misc_feature 1..41: note = Synthetic oligonucleotide (Primary Indication: Alzheimer's Disease; Target: APOE)
  source 1..41: mol_type = other DNA
atgccgatgacctgcagaagtgcctggcagtgtaccaggcc

SEQ ID NO: 81 - DNA, 41 bp, synthetic construct
  misc_feature 1..41: note = Synthetic oligonucleotide (Primary Indication: Alzheimer's Disease; Target: APOE)
  source 1..41: mol_type = other DNA
ggcctggtacactgccaggcacttctgcaggtcatcggcat

SEQ ID NO: 82 - DNA, 179 bp, synthetic construct
  misc_feature 1..179: note = Synthetic oligonucleotide (Primary Indication: Alzheimer's Disease; Target: APOE)
  source 1..179: mol_type = other DNA
gcgcggacatggaggacgtgtgcggccgcctggtgcagtaccgcggcgaggtgcaggccatgctcggccagagcaccgaggagctgcgggtgcgcctcgcctcccacctgcgcaagctgcgtaagcggctcctccgcgatgccgatgacctgcagaagcgcctggcagtgtaccaggcc

SEQ ID NO: 83 - DNA, 179 bp, synthetic construct
  misc_feature 1..179: note = Synthetic oligonucleotide (Primary Indication: Alzheimer's Disease; Target: APOE)
  source 1..179: mol_type = other DNA
ggcctggtacactgccaggcgcttctgcaggtcatcggcatcgcggaggagccgcttacgcagcttgcgcaggtgggaggcgaggcgcacccgcagctcctcggtgctctggccgagcatggcctgcacctcgccgcggtactgcaccaggcggccgcacacgtcctccatgtccgcgc

SEQ ID NO: 84 - DNA, 179 bp, synthetic construct
  misc_feature 1..179: note = Synthetic oligonucleotide (Primary Indication: Alzheimer's Disease; Target: APOE)
  source 1..179: mol_type = other DNA
gcgcggacatggaggacgtgtgcggccgcctggtgcagtaccgcggcgaggtgcaggccatgctcggccagagcaccgaggagctgcgggtgcgcctcgcctcccacctgcgcaagctgcgtaagcggctcctccgcgatgccgatgacctgcagaagtgcctggcagtgtaccaggcc

SEQ ID NO: 85 - DNA, 179 bp, synthetic construct
  misc_feature 1..179: note = Synthetic oligonucleotide (Primary Indication: Alzheimer's Disease; Target: APOE)
  source 1..179: mol_type = other DNA
ggcctggtacactgccaggcacttctgcaggtcatcggcatcgcggaggagccgcttacgcagcttgcgcaggtgggaggcgaggcgcacccgcagctcctcggtgctctggccgagcatggcctgcacctcgccgcggtactgcaccaggcggccgcacacgtcctccatgtccgcgc

SEQ ID NO: 86 - DNA, 70 bp, synthetic construct
  misc_feature 1..70: note = Synthetic oligonucleotide (Primary Indication: Hemophilia A; Target: F8)
  source 1..70: mol_type = other DNA
accgaagctggtacctcacagagaatatacaacgctttctccccaatccagctggagtgcagcttgagga

SEQ ID NO: 87 - DNA, 70 bp, synthetic construct
  misc_feature 1..70: note = Synthetic oligonucleotide (Primary Indication: Hemophilia A; Target: F8)
  source 1..70: mol_type = other DNA
tcctcaagctgcactccagctggattggggagaaagcgttgtatattctctgtgaggtaccagcttcggt

SEQ ID NO: 88 - DNA, 40 bp, synthetic construct
  misc_feature 1..40: note = Synthetic oligonucleotide (Primary Indication: Hemophilia A; Target: F8)
  source 1..40: mol_type = other DNA
acctcacagagaatatacaacgctttctccccaatccagc

SEQ ID NO: 89 - DNA, 40 bp, synthetic construct
  misc_feature 1..40: note = Synthetic oligonucleotide (Primary Indication: Hemophilia A; Target: F8)
  source 1..40: mol_type = other DNA
gctggattggggagaaagcgttgtatattctctgtgaggt

SEQ ID NO: 90 - DNA, 71 bp, synthetic construct
  misc_feature 1..71: note = Synthetic oligonucleotide (Primary Indication: Hemophilia B; Target: F9)
  source 1..71: mol_type = other DNA
agttcttcagtaccttagagttccacttgttgaccgagccacatgtcttcgatctacaaagttcaccatct

SEQ ID NO: 91 - DNA, 71 bp, synthetic construct
  misc_feature 1..71: note = Synthetic oligonucleotide (Primary Indication: Hemophilia B; Target: F9)
  source 1..71: mol_type = other DNA
agatggtgaactttgtagatcgaagacatgtggctcggtcaacaagtggaactctaaggtactgaagaact

SEQ ID NO: 92 - DNA, 41 bp, synthetic construct
  misc_feature 1..41: note = Synthetic oligonucleotide (Primary Indication: Hemophilia B; Target: F9)
  source 1..41: mol_type = other DNA
tagagttccacttgttgaccgagccacatgtcttcgatcta

SEQ ID NO: 93 - DNA, 41 bp, synthetic construct
  misc_feature 1..41: note = Synthetic oligonucleotide (Primary Indication: Hemophilia B; Target: F9)
  source 1..41: mol_type = other DNA
tagatcgaagacatgtggctcggtcaacaagtggaactcta

SEQ ID NO: 94 - DNA, 72 bp, synthetic construct
  misc_feature 1..72: note = Synthetic oligonucleotide (Primary Indication: Sickle cell anemia ; Target: HBB)
  source 1..72: mol_type = other DNA
aacctcaaacagacaccatggtgcatctgactcctgaggagaagtctgccgttactgccctgtggggcaagg

SEQ ID NO: 95 - DNA, 72 bp, synthetic construct
  misc_feature 1..72: note = Synthetic oligonucleotide (Primary Indication: Sickle cell anemia ; Target: HBB)
  source 1..72: mol_type = other DNA
ccttgccccacagggcagtaacggcagacttctcctcaggagtcagatgcaccatggtgtctgtttgaggtt

SEQ ID NO: 96 - DNA, 40 bp, synthetic construct
  misc_feature 1..40: note = Synthetic oligonucleotide (Primary Indication: Sickle cell anemia ; Target: HBB)
  source 1..40: mol_type = other DNA
catggtgcatctgactcctgaggagaagtctgccgttact

SEQ ID NO: 97 - DNA, 40 bp, synthetic construct
  misc_feature 1..40: note = Synthetic oligonucleotide (Primary Indication: Sickle cell anemia ; Target: HBB)
  source 1..40: mol_type = other DNA
agtaacggcagacttctcctcaggagtcagatgcaccatg

SEQ ID NO: 98 - DNA, 71 bp, synthetic construct
  misc_feature 1..71: note = Synthetic oligonucleotide (Primary Indication: TTR Amyloidosis; Target: TTR)
  source 1..71: mol_type = other DNA
atgctgtccgaggcagtcctgccatcaatgtggccgtgcatgtgttcagaaaggctgctgatgacacctgg

SEQ ID NO: 99 - DNA, 71 bp, synthetic construct
  misc_feature 1..71: note = Synthetic oligonucleotide (Primary Indication: TTR Amyloidosis; Target: TTR)
  source 1..71: mol_type = other DNA
ccaggtgtcatcagcagcctttctgaacacatgcacggccacattgatggcaggactgcctcggacagcat

SEQ ID NO: 100 - DNA, 41 bp, synthetic construct
  misc_feature 1..41: note = Synthetic oligonucleotide (Primary Indication: TTR Amyloidosis; Target: TTR)
  source 1..41: mol_type = other DNA
gtcctgccatcaatgtggccgtgcatgtgttcagaaaggct

SEQ ID NO: 101 - DNA, 41 bp, synthetic construct
  misc_feature 1..41: note = Synthetic oligonucleotide (Primary Indication: TTR Amyloidosis; Target: TTR)
  source 1..41: mol_type = other DNA
agcctttctgaacacatgcacggccacattgatggcaggac

SEQ ID NO: 102 - DNA, 40 bp, synthetic construct
  misc_feature 1..40: note = Synthetic oligonucleotide (Primary Indication: Duchenne Musc. Dys.; Target: Dystrophin)
  source 1..40: mol_type = other DNA
caaaaacccaaaatattttggctcctactcagactgttac

SEQ ID NO: 103 - DNA, 40 bp, synthetic construct
  misc_feature 1..40: note = Synthetic oligonucleotide (Primary Indication: Duchenne Musc. Dys.; Target: Dystrophin)
  source 1..40: mol_type = other DNA
gtaacagtctgagtaggagccaaaatattttgggtttttg

SEQ ID NO: 104 - DNA, 70 bp, synthetic construct
  misc_feature 1..70: note = Synthetic oligonucleotide (Primary Indication: Duchenne Musc. Dys.; Target: Dystrophin)
  source 1..70: mol_type = other DNA
cttttttcctttttgcaaaaacccaaaatattttggctcctactcagactgttactctggtgacacaacc

SEQ ID NO: 105 - DNA, 70 bp, synthetic construct
  misc_feature 1..70: note = Synthetic oligonucleotide (Primary Indication: Duchenne Musc. Dys.; Target: Dystrophin)
  source 1..70: mol_type = other DNA
ggttgtgtcaccagagtaacagtctgagtaggagccaaaatattttgggtttttgcaaaaaggaaaaaag

SEQ ID NO: 106 - DNA, 71 bp, synthetic construct
  misc_feature 1..71: note = Synthetic oligonucleotide (Primary Indication: Cystic Fibrosis; Target: CFTR)
  source 1..71: mol_type = other DNA
ggattatgcctggcaccattaaagaaaatatcatctttggtgtttcctatgatgaatatagatacagaagc

SEQ ID NO: 107 - DNA, 71 bp, synthetic construct
  misc_feature 1..71: note = Synthetic oligonucleotide (Primary Indication: Cystic Fibrosis; Target: CFTR)
  source 1..71: mol_type = other DNA
gcttctgtatctatattcatcataggaaacaccaaagatgatattttctttaatggtgccaggcataatcc

SEQ ID NO: 108 - DNA, 41 bp, synthetic construct
  misc_feature 1..41: note = Synthetic oligonucleotide (Primary Indication: Cystic Fibrosis; Target: CFTR)
  source 1..41: mol_type = other DNA
ccattaaagaaaatatcatctttggtgtttcctatgatgaa

SEQ ID NO: 109 - DNA, 41 bp, synthetic construct
  misc_feature 1..41: note = Synthetic oligonucleotide (Primary Indication: Cystic Fibrosis; Target: CFTR)
  source 1..41: mol_type = other DNA
ttcatcataggaaacaccaaagatgatattttctttaatgg

SEQ ID NO: 110 - DNA, 61 bp, synthetic construct
  misc_feature 1..61: note = Synthetic oligonucleotide (Primary Indication: Cystic Fibrosis; Target: CFTR)
  source 1..61: mol_type = other DNA
ttctgtatctatattcatcataggaaacaccaaagataatgttctccttaatggtgccagg